European Patent Specification EP 3 555 128 B1, published December 27, 2023. Title: ANTI-PCNA MONOCLONAL ANTIBODIES AND USE THEREOF. Applicant: National institute for biotechnology of the negev. The sequence listing filed with the application follows.

SEQUENCE LISTING (35 sequences)

SEQ ID NO: 1 - protein, 6 aa, Artificial Sequence
  Synthetic
GFSFNI

SEQ ID NO: 2 - protein, 12 aa, Artificial Sequence
  Synthetic
RIRSKSNNYATY

SEQ ID NO: 3 - protein, 13 aa, Artificial Sequence
  Synthetic
HPNYSGFNYPFAS

SEQ ID NO: 4 - protein, 16 aa, Artificial Sequence
  Synthetic
RSSQSIVHSNGKTYFE

SEQ ID NO: 5 - protein, 7 aa, Artificial Sequence
  Synthetic
KVSNRFS

SEQ ID NO: 6 - protein, 9 aa, Artificial Sequence
  Synthetic
FQGSHVPYT

SEQ ID NO: 7 - protein, 122 aa, Artificial Sequence
  Synthetic
KLVESGGGLVQPTGSLKLSCVTSGFSFNIYAMNWVRQAPGKGLEWVARIRSKSNNYATYYADSVKDRFTISRDDSESMLYLQMNNLKTEDTAMYYCMRHPNYSGFNYPFASWGPGTLVTVSA

SEQ ID NO: 8 - protein, 112 aa, Artificial Sequence
  Synthetic
DVVMTQTPLSLPVSLGDQASISCRSSQSIVHSNGKTYFEWYLQKPGQSPKLLIYKVSNRFSGVPDRFSGSGSGTEFTLKISRVEAEDLGVYYCFQGSHVPYTFGGGTKLEIK

SEQ ID NO: 9 - protein, 324 aa, Artificial Sequence
  Synthetic
AKTTPPSVYPLAPGSAAQTNSMVTLGCLVKGYFPEPVTVTWNSGSLSSGVHTFPAVLQSDLYTLSSSVTVPSSTWPSQTVTCNVAHPASSTKVDKKIVPRDCGCKPCICTVPEVSSVFIFPPKPKDVLTITLTPKVTCVVVDISKDDPEVQFSWFVDDVEVHTAQTKPREEQINSTFRSVSELPIMHQDWLNGKEFKCRVNSAAFPAPIEKTISKTKGRPKAPQVYTIPPPKEQMAKDKVSLTCMITNFFPEDITVEWQWNGQPAENYKNTQPIMDTDGSYFVYSKLNVQKSNWEAGNTFTCSVLHEGLHNHHTEKSLSHSPGK

SEQ ID NO: 10 - protein, 107 aa, Artificial Sequence
  Synthetic
RADAAPTVSIFPPSSEQLTSGGASVVCFLNNFYPKDINVKWKIDGSERQNGVLNSWTDQDSKDSTYSMSSTLTLTKDEYERHNSYTCEATHKTSTSPIVKSFNRNEC

SEQ ID NO: 11 - protein, 6 aa, Artificial Sequence
  Synthetic
VYAFSS

SEQ ID NO: 12 - protein, 10 aa, Artificial Sequence
  Synthetic
RIYPADGDTN

SEQ ID NO: 13 - protein, 7 aa, Artificial Sequence
  Synthetic
WLRAMDY

SEQ ID NO: 14 - protein, 11 aa, Artificial Sequence
  Synthetic
KASQNVGTNVA

SEQ ID NO: 15 - protein, 7 aa, Artificial Sequence
  Synthetic
SASYRYS

SEQ ID NO: 16 - protein, 9 aa, Artificial Sequence
  Synthetic
QQYNSYPYT

SEQ ID NO: 17 - protein, 104 aa, Artificial Sequence
  Synthetic
EPGASVKISCKASVYAFSSSWMNWVKQRPGKGLEWIGRIYPADGDTNYNGNFRGKATLTADKSSSTAYMQLSSLTSEDSAVYFCARWLRAMDYWGQGTSVTVSS

SEQ ID NO: 18 - protein, 107 aa, Artificial Sequence
  Synthetic
DIVMTQSQKIMSTSVGDRVSVTCKASQNVGTNVAWYQQKPGQSPKVLIYSASYRYSGVPDRFTGSGSGTDFTLSISNVQSEDLAEYFCQQYNSYPYTFGGGTKLEIK

SEQ ID NO: 19 - protein, 325 aa, Artificial Sequence
  Synthetic
AKTTYPPSVYPLAPGSAAQTNSMVTLGCLVKGYFPEPVTVTWNSGSLSSGVHTFPAVLQSDLYTLSSSVTVPSSTWPSETVTCNVAHPASSTKVDKKIVPRDCGCKPCICTVPEVSSVFIFPPKPKDVLTITLTPKVTCVVVDISKDDPEVQFSWFVDDVEVHTAQTQPREEQFNSTFRSVSELPIMHQDWLNGKEFKCRVNSAAFPAPIEKTISKTKGRPKAPQVYTIPPPKEQMAKDKVSLTCMITDFFPEDITVEWQWNGQPAENYKNTQPIMDTDGSYFVYSKLNVQKSNWEAGNTFTCSVLHEGLHNHHTEKSLSHSPGK

SEQ ID NO: 20 - protein, 107 aa, Artificial Sequence; identical to SEQ ID NO: 10
  Synthetic

SEQ ID NO: 21 - protein, 5 aa, Artificial Sequence
  Synthetic
IYAMN

SEQ ID NO: 22 - protein, 10 aa, Artificial Sequence
  Synthetic
GFSFNIYAMN

SEQ ID NO: 23 - protein, 19 aa, Artificial Sequence
  Synthetic
RIRSKSNNYATYYADSVKD

SEQ ID NO: 24 - protein, 5 aa, Artificial Sequence
  Synthetic
SSWMN

SEQ ID NO: 25 - protein, 10 aa, Artificial Sequence
  Synthetic
VYAFSSSWMN

SEQ ID NO: 26 - protein, 17 aa, Artificial Sequence
  Synthetic
RIYPADGDTNYNGNFRG

SEQ ID NO: 27 - DNA, 322 bp, Artificial Sequence
  Synthetic
tgacattgtgatgactcagtctcaaaaaatcatgtccacatcagtaggagacagggtcagcgtcacctgcaaggccagtcagaatgtgggtactaatgtagcctggtatcaacagaaaccagggcaatctcctaaagtactgatttactcggcatcctaccggtacagtggagtccctgatcgcttcacaggcagtggatctgggacagatttcactctcagcatcagcaatgtgcagtctgaagacttggcagagtatttctgtcagcaatataacagctatccgtacacgttcggaggggggaccaagctggaaataaaa

SEQ ID NO: 28 - DNA, 325 bp, Artificial Sequence
  Synthetic
cgggctgatgctgcaccaactgtatccatcttcccaccatccagtgagcagttaacatctggaggtgcctcagtcgtgtgcttcttgaacaacttctaccccaaagacatcaatgtcaagtggaagattgatggcagtgaacgacaaaatggcgtcctgaacagttggactgatcaggacagcaaagacagcacctacagcatgagcagcaccctcacgttgaccaaggacgagtatgaacgacataacagctatacctgtgaggccactcacaagacatcaacttcacccattgtcaagagcttcaacaggaatgagtgttaga

SEQ ID NO: 29 - DNA, 312 bp, Artificial Sequence
  Synthetic
gagcctggggcctcagtgaagatttcctgcaaggcttctgtctacgcattcagtagttcctggatgaactgggtgaagcagaggcctggaaagggtcttgagtggattggacggatttatcctgcagatggagatactaactacaatgggaacttcaggggcaaggccacactgactgcagacaaatcctccagcacagcctacatgcaactcagcagtctgacatctgaggactctgcggtctacttctgtgcaagatggttacgggctatggactactggggtcaaggaacctcagtcaccgtctcctca

SEQ ID NO: 30 - DNA, 978 bp, Artificial Sequence
  Synthetic
gccaaaacaacataccccccatctgtctatccactggcccctggatctgctgcccaaactaactccatggtgaccctgggatgcctggtcaagggctatttccctgagccagtgacagtgacctggaactctggatccctgtccagcggtgtgcacaccttcccagctgtcctgcagtctgacctctacactctgagcagctcagtgactgtcccctccagcacctggcccagcgagaccgtcacctgcaacgttgcccacccggccagcagcaccaaggtggacaagaaaattgtgcccagggattgtggttgtaagccttgcatatgtacagtcccagaagtatcatctgtcttcatcttccccccaaagcccaaggatgtgctcaccattactctgactcctaaggtcacgtgtgttgtggtagacatcagcaaggatgatcccgaggtccagttcagctggtttgtagatgatgtggaggtgcacacagctcagacgcaaccccgggaggagcagttcaacagcactttccgctcagtcagtgaacttcccatcatgcaccaggactggctcaatggcaaggagttcaaatgcagggtcaacagtgcagctttccctgcccccatcgagaaaaccatctccaaaaccaaaggcagaccgaaggctccacaggtgtacaccattccacctcccaaggagcagatggccaaggataaagtcagtctgacctgcatgataacagacttcttccctgaagacattactgtggagtggcagtggaatgggcagccagcggagaactacaagaacactcagcccatcatggacacagatggctcttacttcgtctacagcaagctcaatgtgcagaagagcaactgggaggcaggaaatactttcacctgctctgtgttacatgagggcctgcacaaccaccatactgagaagagcctctcccactctcctggtaaatga

SEQ ID NO: 31 - DNA, 337 bp, Artificial Sequence
  Synthetic
tgatgttgtgatgacccaaactccgctctccctgcctgtcagtcttggagatcaagcctccatctcttgcagatctagtcagagcattgtacatagtaatggaaagacctattttgaatggtaccttcagaaaccaggccagtctccaaagctcctgatctacaaagtttccaaccgattttctggggtcccagacaggttcagtggcagtggatcagggacagaattcacactcaagatcagcagagtggaggctgaggatctgggagtttattactgctttcaaggttcacatgttccgtacacgttcggaggggggaccaagctggaaataaaa

SEQ ID NO: 32 - DNA, 324 bp, Artificial Sequence
  Synthetic
cgggctgatgctgcaccaactgtatccatcttcccaccatccagtgagcagttaacatctggaggtgcctcagtcgtgtgcttcttgaacaacttctaccccaaagacatcaatgtcaagtggaagattgatggcagtgaacgacaaaatggcgtcctgaacagttggactgatcaggacagcaaagacagcacctacagcatgagcagcaccctcacgttgaccaaggacgagtatgaacgacataacagctatacctgtgaggccactcacaagacatcaacttcacccattgtcaagagcttcaacaggaatgagtgttag

SEQ ID NO: 33 - DNA, 366 bp, Artificial Sequence
  Synthetic
aagctggtggagtctggtggaggattggtgcagcctacagggtcattgaaactctcatgtgtaacctctggattcagtttcaatatctacgccatgaactgggtccgccaggctccaggaaagggtttggaatgggttgctcgcataagaagtaaaagtaataattatgcaacatattatgccgattcagtgaaagacagattcaccatctccagagatgattcagaaagcatgctctatctccaaatgaacaacttgaaaactgaggacacagccatgtattactgtatgagacaccccaattactccggctttaactacccgtttgcttcctggggcccagggactctggtcactgtctctgca

SEQ ID NO: 34 - DNA, 975 bp, Artificial Sequence
  Synthetic
gccaaaacgacacccccatctgtctatccactggcccctggatctgctgcccaaactaactccatggtgaccctgggatgcctggtcaagggctatttccctgagccagtgacagtgacctggaactctggatccctgtccagcggtgtgcacaccttcccagctgtcctgcagtctgacctctacactctgagcagctcagtgactgtcccctccagcacctggcccagccagaccgtcacctgcaacgttgcccacccggccagcagcaccaaggtggacaagaaaattgtgcccagggattgtggttgtaagccttgcatatgtacagtcccagaagtatcatctgtcttcatcttccccccaaagcccaaggatgtgctcaccattactctgactcctaaggtcacgtgtgttgtggtagacatcagcaaggatgatcccgaggtccagttcagctggtttgtagatgatgtggaggtgcacacagctcagacgaaaccccgggaggagcagatcaacagcactttccgttcagtcagtgaacttcccatcatgcaccaggactggctcaatggcaaggagttcaaatgcagggtcaacagtgcagctttccctgcccccatcgagaaaaccatctccaaaaccaaaggcagaccgaaggctccacaggtgtacaccattccacctcccaaggagcagatggccaaggataaagtcagtctgacctgcatgataacaaacttcttccctgaagacattactgtggagtggcagtggaatgggcagccagcggagaactacaagaacactcagcccatcatggacacagatggctcttacttcgtctacagcaagctcaatgtgcagaagagcaactgggaggcaggaaatactttcacctgctctgtgttacatgagggcctgcacaaccaccatactgagaagagcctctcccactctcctggtaaatga

SEQ ID NO: 35 - protein, 276 aa, Homo sapiens
MAWRALHPLLLLLLLFPGSQAQSKAQVLQSVAGQTLTVRCQYPPTGSLYEKKGWCKEASALVCIRLVTSSKPRTMAWTSRFTIWDDPDAGFFTVTMTDLREEDSGHYWCRIYRPSDNSVSKSVRFYLVVSPASASTQTSWTPRDLVSSQTQTQSCVPPTAGARQAPESPSTIPVPSQPQNSTLRPGPAAPIALVPVFCGLLVAKSLVLSALLVWWGDIWWKTMMELRSLDTQKATCHLQQVTDLPWTSVSSPVEREILYHTVARTKISDDDDEHTL